European Patent Application EP 4 365 204 A1, published May 8, 2024. Title: Methods for preparing a sample comprising circulating tumor cells in blood. Applicant: Novacellum Inc. The sequence listing filed with the application follows.

SEQUENCE LISTING (98 sequences)

SEQ ID NO: 1 - protein, 9 aa, Homo sapiens
MAAVGVSSV

SEQ ID NO: 2 - protein, 8 aa, Homo sapiens
RYIYRVLL

SEQ ID NO: 3 - protein, 9 aa, Homo sapiens
PWADFSFKF

SEQ ID NO: 4 - protein, 9 aa, Homo sapiens
FSFKFMPQV

SEQ ID NO: 5 - protein, 9 aa, Homo sapiens
TWLFNSRKW

SEQ ID NO: 6 - protein, 9 aa, Homo sapiens
AQWGHVHSL

SEQ ID NO: 7 - protein, 9 aa, Homo sapiens
TFSNYGMHW

SEQ ID NO: 8 - protein, 9 aa, Homo sapiens
MAHCILDLL

SEQ ID NO: 9 - protein, 9 aa, Homo sapiens
TLKELFFRL

SEQ ID NO: 10 - protein, 10 aa, Homo sapiens
FMPQVYVPTT

SEQ ID NO: 11 - protein, 9 aa, Homo sapiens
CLCPHPPAA

SEQ ID NO: 12 - protein, 9 aa, Homo sapiens
WADFSFKFM

SEQ ID NO: 13 - protein, 9 aa, Homo sapiens
AQWGHVHSL

SEQ ID NO: 14 - protein, 9 aa, Homo sapiens
FMPQVYVPT

SEQ ID NO: 15 - protein, 11 aa, Homo sapiens
FLGTEDLYDYI

SEQ ID NO: 16 - protein, 10 aa, Homo sapiens
LLIPRPLNPA

SEQ ID NO: 17 - protein, 11 aa, Homo sapiens
LLIPRPLNPAL

SEQ ID NO: 18 - protein, 10 aa, Homo sapiens
KTLKELFFRL

SEQ ID NO: 19 - protein, 11 aa, Homo sapiens
FMPQVYVPTTF

SEQ ID NO: 20 - protein, 9 aa, Homo sapiens
FSNYGMHWV

SEQ ID NO: 21 - protein, 9 aa, Homo sapiens
FSFKFMPQV

SEQ ID NO: 22 - protein, 10 aa, Homo sapiens
HLHPPGTQEV

SEQ ID NO: 23 - protein, 9 aa, Homo sapiens
RTMRPLPGR

SEQ ID NO: 24 - protein, 9 aa, Homo sapiens
RPLPGRIEV

SEQ ID NO: 25 - protein, 10 aa, Homo sapiens
LQLSQALSLM

SEQ ID NO: 26 - protein, 11 aa, Homo sapiens
RQAMMEKVRSY

SEQ ID NO: 27 - protein, 9 aa, Homo sapiens
KVQLDSSHR

SEQ ID NO: 28 - protein, 10 aa, Homo sapiens
RPLPGRIEVR

SEQ ID NO: 29 - protein, 10 aa, Homo sapiens
RTMRPLPGRI

SEQ ID NO: 30 - protein, 9 aa, Homo sapiens
ALLQLSQAL

SEQ ID NO: 31 - protein, 20 aa, Homo sapiens
RQAMMEKVRSYGSVLLSAEE

SEQ ID NO: 32 - protein, 20 aa, Homo sapiens
HRQAMMEKVRSYGSVLLSAE

SEQ ID NO: 33 - protein, 20 aa, Homo sapiens
SHRQAMMEKVRSYGSVLLSA

SEQ ID NO: 34 - protein, 25 aa, Homo sapiens
HRQAMMEKVRSYGSVLLSAEEFQKL

SEQ ID NO: 35 - protein, 25 aa, Homo sapiens
SHRQAMMEKVRSYGSVLLSAEEFQK

SEQ ID NO: 36 - protein, 24 aa, Homo sapiens
RQAMMEKVRSYGSVLLSAEEFQKL

SEQ ID NO: 37 - protein, 24 aa, Homo sapiens
HRQAMMEKVRSYGSVLLSAEEFQK

SEQ ID NO: 38 - protein, 25 aa, Homo sapiens
SSHRQAMMEKVRSYGSVLLSAEEFQ

SEQ ID NO: 39 - protein, 9 aa, Homo sapiens
AAQERRLQL

SEQ ID NO: 40 - protein, 10 aa, Homo sapiens
TTHPTHVPSF

SEQ ID NO: 41 - protein, 9 aa, Homo sapiens
QLQSPLLGR

SEQ ID NO: 42 - protein, 10 aa, Homo sapiens
GQEFADFEYR

SEQ ID NO: 43 - protein, 10 aa, Homo sapiens
VQLQSPLLGR

SEQ ID NO: 44 - protein, 15 aa, Homo sapiens
LDAVQLQSPLLGRLW

SEQ ID NO: 45 - protein, 15 aa, Homo sapiens
LLDAVQLQSPLLGRL

SEQ ID NO: 46 - protein, 17 aa, Homo sapiens
SLLDAVQLQSPLLGRLW

SEQ ID NO: 47 - protein, 17 aa, Homo sapiens
LLDAVQLQSPLLGRLWL

SEQ ID NO: 48 - protein, 15 aa, Homo sapiens
DAVQLQSPLLGRLWL

SEQ ID NO: 49 - protein, 11 aa, Homo sapiens
REDRASAPAAL

SEQ ID NO: 50 - protein, 10 aa, Homo sapiens
REQASGWGGL

SEQ ID NO: 51 - protein, 9 aa, Homo sapiens
LQDDVFPEH

SEQ ID NO: 52 - protein, 9 aa, Homo sapiens
GELLSPSHA

SEQ ID NO: 53 - protein, 11 aa, Homo sapiens
LQDDVFPEHAL

SEQ ID NO: 54 - protein, 9 aa, Homo sapiens
RLGEKPAAA

SEQ ID NO: 55 - protein, 9 aa, Homo sapiens
RLGEKPAAA

SEQ ID NO: 56 - protein, 10 aa, Homo sapiens
STAPVTATSF

SEQ ID NO: 57 - protein, 20 aa, Homo sapiens
GGYRDKMRMQKTQLSPEIKV

SEQ ID NO: 58 - protein, 20 aa, Homo sapiens
QGGYRDKMRMQKTQLSPEIK

SEQ ID NO: 59 - protein, 20 aa, Homo sapiens
GYRDKMRMQKTQLSPEIKVC

SEQ ID NO: 60 - protein, 20 aa, Homo sapiens
AQGGYRDKMRMQKTQLSPEI

SEQ ID NO: 61 - protein, 20 aa, Homo sapiens
YRDKMRMQKTQLSPEIKVCQ

SEQ ID NO: 62 - protein, 15 aa, Homo sapiens
RDKMRMQKTQLSPEI

SEQ ID NO: 63 - protein, 25 aa, Homo sapiens
QAQGGYRDKMRMQKTQLSPEIKVCQ

SEQ ID NO: 64 - protein, 25 aa, Homo sapiens
LQAQGGYRDKMRMQKTQLSPEIKVC

SEQ ID NO: 65 - protein, 8 aa, Homo sapiens
LCPMQRFL

SEQ ID NO: 66 - protein, 11 aa, Homo sapiens
EFKEKPDMSRF

SEQ ID NO: 67 - protein, 9 aa, Homo sapiens
KLAGGLCPM

SEQ ID NO: 68 - protein, 25 aa, Homo sapiens
KAAVGEEKDINTFLGTPVQKLDQPG

SEQ ID NO: 69 - protein, 25 aa, Homo sapiens
PKAAVGEEKDINTFLGTPVQKLDQP

SEQ ID NO: 70 - protein, 25 aa, Homo sapiens
TPKAAVGEEKDINTFLGTPVQKLDQ

SEQ ID NO: 71 - protein, 19 aa, Homo sapiens
AAVGEEKDINTFLGTPVQK

SEQ ID NO: 72 - protein, 9 aa, Homo sapiens
FLVAFLEGV

SEQ ID NO: 73 - protein, 9 aa, Homo sapiens
TQSSDSLAV

SEQ ID NO: 74 - protein, 9 aa, Homo sapiens
FLEGVQCEV

SEQ ID NO: 75 - protein, 9 aa, Homo sapiens
YILQEGDLV

SEQ ID NO: 76 - protein, 9 aa, Homo sapiens
RWVFLVAFL

SEQ ID NO: 77 - protein, 9 aa, Homo sapiens
LQEGDLVKI

SEQ ID NO: 78 - protein, 10 aa, Homo sapiens
QLLESGGDLV

SEQ ID NO: 79 - protein, 9 aa, Homo sapiens
QSISTWLAW

SEQ ID NO: 80 - protein, 9 aa, Homo sapiens
RASQSISTW

SEQ ID NO: 81 - protein, 11 aa, Homo sapiens
ASQSISTWLAW

SEQ ID NO: 82 - protein, 9 aa, Homo sapiens
LTLTGFATA

SEQ ID NO: 83 - protein, 10 aa, Homo sapiens
ISSLLTLTGF

SEQ ID NO: 84 - protein, 9 aa, Homo sapiens
SSLLTLTGF

SEQ ID NO: 85 - protein, 11 aa, Homo sapiens
SLLTLTGFATA

SEQ ID NO: 86 - protein, 9 aa, Homo sapiens
AVLQAHYAK

SEQ ID NO: 87 - protein, 9 aa, Homo sapiens
SAYSGNTNY

SEQ ID NO: 88 - protein, 11 aa, Homo sapiens
AVAVLQAHYAK

SEQ ID NO: 89 - protein, 10 aa, Homo sapiens
AVLQAHYAKK

SEQ ID NO: 90 - protein, 9 aa, Homo sapiens
AVLQAHYAK

SEQ ID NO: 91 - protein, 9 aa, Homo sapiens
SLAMSLGER

SEQ ID NO: 92 - protein, 9 aa, Homo sapiens
VLQAHYAKK

SEQ ID NO: 93 - protein, 10 aa, Homo sapiens
VAVLQAHYAK

SEQ ID NO: 94 - protein, 10 aa, Homo sapiens
QVESGGGLVK

SEQ ID NO: 95 - protein, 9 aa, Homo sapiens
SAYSGNTNY

SEQ ID NO: 96 - protein, 10 aa, Homo sapiens
YSGNTNYAQK

SEQ ID NO: 97 - protein, 10 aa, Homo sapiens
RSNPFNESQK

SEQ ID NO: 98 - protein, 11 aa, Homo sapiens
RSNPFNESQKK